European Patent Specification EP 4 305 201 B1, published September 9, 2026. Title: CHEMICAL SAMPLE INDEXING FOR HIGH-THROUGHPUT SINGLE-CELL ANALYSIS. Applicant: Singleron (Nanjing) Biotechnologies, Ltd. Nanjing University. The sequence listing filed with the application follows.

SEQUENCE LISTING (1 sequence)

SEQ ID NO: 1 - DNA, 59 bp, Artificial Sequence
  Synthetic Oligonucleotide
tgtcaagatgctaccgttcagagtgacctgcttcacgcaaaaaaaaaaaaaaaaaaaaa